European Patent Specification EP 3 938 541 B9, published October 4, 2023. Title: METHOD FOR SEQUENCING A DIRECT REPEAT. Applicant: Genome Research Limited. The sequence listing filed with the application follows.

SEQUENCE LISTING (3 sequences)

SEQ ID NO: 1 - DNA, 11 bp, artificial sequence
  synthetic oligonucleotide
gatcggatcga

SEQ ID NO: 2 - DNA, 11 bp, artificial sequence
  sythetic oligonucleotide
gatcgtatcga

SEQ ID NO: 3 - DNA, 12 bp, artificial sequence
  synthetic oligonucleotide
  misc_feature (7)..(7): n at position 7 is a G or T
gatcggnatcga